European Patent Application EP 4 741 414 A1, published May 13, 2026. Title: Peptide having cell membrane permeability and screening method therefor. Applicant: MeSCue-Janusys Inc. Application JP. The sequence listing filed with the application follows.

SEQUENCE LISTING (56 sequences)

SEQ ID NO: 1 - protein, 13 aa, synthetic construct
CKMWSPYGQETYC

SEQ ID NO: 2 - protein, 12 aa, synthetic construct
CNRYRMIVDQSC

SEQ ID NO: 3 - protein, 11 aa, synthetic construct
CSKNWYGWMFC

SEQ ID NO: 4 - protein, 10 aa, synthetic construct
FQIYKFAFMV

SEQ ID NO: 5 - protein, 10 aa, synthetic construct
GWKIPYLWHV

SEQ ID NO: 6 - protein, 10 aa, synthetic construct
GYYKRMIKQQ

SEQ ID NO: 7 - protein, 10 aa, synthetic construct
LFKAWLGVYH

SEQ ID NO: 8 - protein, 10 aa, synthetic construct
MNYHKSNRHN

SEQ ID NO: 9 - protein, 10 aa, synthetic construct
RVVSYLAEYH

SEQ ID NO: 10 - protein, 10 aa, synthetic construct
VDMKSSNRLW

SEQ ID NO: 11 - protein, 10 aa, synthetic construct
YFDDWLAPYH

SEQ ID NO: 12 - protein, 14 aa, synthetic construct
CIRYYVARHVRRRC

SEQ ID NO: 13 - protein, 11 aa, synthetic construct
CRMAPQFNHVC

SEQ ID NO: 14 - protein, 10 aa, synthetic construct
RVVSYLAEYQ

SEQ ID NO: 15 - protein, 10 aa, synthetic construct
TVTRGERYKH

SEQ ID NO: 16 - protein, 10 aa, synthetic construct
VHSWVDMAKN

SEQ ID NO: 17 - protein, 10 aa, synthetic construct
YVDDWLAPYH

SEQ ID NO: 18 - protein, 10 aa, synthetic construct
QYNMVRQDLI

SEQ ID NO: 19 - protein, 10 aa, synthetic construct
VRVKTYWENH

SEQ ID NO: 20 - protein, 12 aa, synthetic construct
FLPMFSRLGLQI

SEQ ID NO: 21 - protein, 12 aa, synthetic construct
FSVRLPMFSFRL

SEQ ID NO: 22 - protein, 10 aa, synthetic construct
IQIKVMAWLT

SEQ ID NO: 23 - protein, 10 aa, synthetic construct
KWPVINVEVK

SEQ ID NO: 24 - protein, 10 aa, synthetic construct
LFARLLDMFF

SEQ ID NO: 25 - protein, 10 aa, synthetic construct
LYARILNWIF

SEQ ID NO: 26 - protein, 10 aa, synthetic construct
LYHTAIKTFT

SEQ ID NO: 27 - protein, 10 aa, synthetic construct
QALLKLYFSF

SEQ ID NO: 28 - protein, 12 aa, synthetic construct
RLIFRHVIDMIF

SEQ ID NO: 29 - protein, 10 aa, synthetic construct
VHVHVMINFF

SEQ ID NO: 30 - protein, 10 aa, synthetic construct
WYMVHLRSEW

SEQ ID NO: 31 - protein, 10 aa, synthetic construct
SHYSLIVFSR

SEQ ID NO: 32 - protein, 14 aa, synthetic construct
CHMVNTYKWTFFIC

SEQ ID NO: 33 - protein, 14 aa, synthetic construct
CTPWKNRNVLLWYC

SEQ ID NO: 34 - protein, 10 aa, synthetic construct
HFHYYMHSVY

SEQ ID NO: 35 - protein, 10 aa, synthetic construct
KILIFHYIFV

SEQ ID NO: 36 - protein, 10 aa, synthetic construct
RWLIFHYMLL

SEQ ID NO: 37 - protein, 10 aa, synthetic construct
RWPLWMWFVW

SEQ ID NO: 38 - protein, 10 aa, synthetic construct
RYYAHWLHYM

SEQ ID NO: 39 - protein, 10 aa, synthetic construct
YYLLPLHVKH

SEQ ID NO: 40 - protein, 10 aa, synthetic construct
RWNCVSCAFL

SEQ ID NO: 41 - DNA, 1001 bp, synthetic construct
  source 1..1001: mol_type = other DNA
gctcttgtcattgtgcttcgcatgattacgaattcagatctcgatcccgcgaaattaatacgactcactatagggagaccacaacggtttccctctagaaataattttgtttaactttaagaaggagatataccaatggtttcaaaaggtgaagaactgttcaccggggtggtgcccatcctggtcgagctggacggcgacgtaaacggccacaagttcagcgtgtccggcgagggcgagggcgatgccacctacggcaagctgaccctgaagttcatctgcaccaccggcaagctgcccgtgccctggcccaccctcgtgaccaccctgacctacggcgtgcagtgcttcagccgctaccccgaccacatgaagcagcacgacttcttcaagtccgccatgcccgaaggctacgtccaggagcgcaccatcttcttcaaggacgacggcaactacaagacccgcgccgaggtgaagttcgagggcgacaccctggtgaaccgcatcgagctgaagggcatcgacttcaaggaggacggcaacatcctggggcacaagctggagtacaactacaacagccacaacgtctatatcatggccgacaagcagaagaacggcatcaaggtgaacttcaagatccgccacaacatcgaggacggcagcgtgcagctcgccgaccactaccagcagaacacccccatcggcgacggccccgtgctgctgcccgacaaccactacctgagcacccagtccgccctgagcaaagaccccaacgagaagcgcgatcacatggtcctgctggagttcgtgaccgccgccgggatcactctcggcatggacgagctgtacaagggtggttcaggttcacatcatcatcatcatcattaataattgattgatctagcataaccccttggggcctctaaacgggtcttgaggggttttttgctgaaaggaggaactatatccggataacctcgagctgcaggcatgcaagcttg

SEQ ID NO: 42 - DNA, 1034 bp, synthetic construct
  source 1..1034: mol_type = other DNA
gctcttgtcattgtgcttcgcatgattacgaattcagatctcgatcccgcgaaattaatacgactcactatagggagaccacaacggtttccctctagaaataattttgtttaactttaagaaggagatataccaatggtttcaaaaggtgaagaactgttcaccggggtggtgcccatcctggtcgagctggacggcgacgtaaacggccacaagttcagcgtgtccggcgagggcgagggcgatgccacctacggcaagctgaccctgaagttcatctgcaccaccggcaagctgcccgtgccctggcccaccctcgtgaccaccctgacctacggcgtgcagtgcttcagccgctaccccgaccacatgaagcagcacgacttcttcaagtccgccatgcccgaaggctacgtccaggagcgcaccatcttcttcaaggacgacggcaactacaagacccgcgccgaggtgaagttcgagggcgacaccctggtgaaccgcatcgagctgaagggcatcgacttcaaggaggacggcaacatcctggggcacaagctggagtacaactacaacagccacaacgtctatatcatggccgacaagcagaagaacggcatcaaggtgaacttcaagatccgccacaacatcgaggacggcagcgtgcagctcgccgaccactaccagcagaacacccccatcggcgacggccccgtgctgctgcccgacaaccactacctgagcacccagtccgccctgagcaaagaccccaacgagaagcgcgatcacatggtcctgctggagttcgtgaccgccgccgggatcactctcggcatggacgagctgtacaagggtggttcatatggtagaaaaaaaagaagacaaagaagaagaggttcacatcatcatcatcatcattaataattgattgatctagcataaccccttggggcctctaaacgggtcttgaggggttttttgctgaaaggaggaactatatccggataacctcgagctgcaggcatgcaagcttg

SEQ ID NO: 43 - DNA, 988 bp, synthetic construct
  source 1..988: mol_type = other DNA
catgattacgaattcagatctcgatcccgcgaaattaatacgactcactatagggagaccacaacggtttccctctagaaataattttgtttaactttaagaaggagatataccaatggtttcaaaaggtgaagaactgttcaccggggtggtgcccatcctggtcgagctggacggcgacgtaaacggccacaagttcagcgtgtccggcgagggcgagggcgatgccacctacggcaagctgaccctgaagttcatctgcaccaccggcaagctgcccgtgccctggcccaccctcgtgaccaccctgacctacggcgtgcagtgcttcagccgctaccccgaccacatgaagcagcacgacttcttcaagtccgccatgcccgaaggctacgtccaggagcgcaccatcttcttcaaggacgacggcaactacaagacccgcgccgaggtgaagttcgagggcgacaccctggtgaaccgcatcgagctgaagggcatcgacttcaaggaggacggcaacatcctggggcacaagctggagtacaactacaacagccacaacgtctatatcatggccgacaagcagaagaacggcatcaaggtgaacttcaagatccgccacaacatcgaggacggcagcgtgcagctcgccgaccactaccagcagaacacccccatcggcgacggccccgtgctgctgcccgacaaccactacctgagcacccagtccgccctgagcaaagaccccaacgagaagcgcgatcacatggtcctgctggagttcgtgaccgccgccgggatcactctcggcatggacgagctgtacaagggtggttcattatttaaagcttggttaggtgtatatcatggttcacatcatcatcatcatcattaataattgattgatctagcataaccccttggggcctctaaacgggtcttgaggggttttttgctgaaaggaggaactatatccggataacct

SEQ ID NO: 44 - DNA, 988 bp, synthetic construct
  source 1..988: mol_type = other DNA
catgattacgaattcagatctcgatcccgcgaaattaatacgactcactatagggagaccacaacggtttccctctagaaataattttgtttaactttaagaaggagatataccaatggtttcaaaaggtgaagaactgttcaccggggtggtgcccatcctggtcgagctggacggcgacgtaaacggccacaagttcagcgtgtccggcgagggcgagggcgatgccacctacggcaagctgaccctgaagttcatctgcaccaccggcaagctgcccgtgccctggcccaccctcgtgaccaccctgacctacggcgtgcagtgcttcagccgctaccccgaccacatgaagcagcacgacttcttcaagtccgccatgcccgaaggctacgtccaggagcgcaccatcttcttcaaggacgacggcaactacaagacccgcgccgaggtgaagttcgagggcgacaccctggtgaaccgcatcgagctgaagggcatcgacttcaaggaggacggcaacatcctggggcacaagctggagtacaactacaacagccacaacgtctatatcatggccgacaagcagaagaacggcatcaaggtgaacttcaagatccgccacaacatcgaggacggcagcgtgcagctcgccgaccactaccagcagaacacccccatcggcgacggccccgtgctgctgcccgacaaccactacctgagcacccagtccgccctgagcaaagaccccaacgagaagcgcgatcacatggtcctgctggagttcgtgaccgccgccgggatcactctcggcatggacgagctgtacaagggtggttcaagagtagtatcatatttagcagaatatcatggttcacatcatcatcatcatcattaataattgattgatctagcataaccccttggggcctctaaacgggtcttgaggggttttttgctgaaaggaggaactatatccggataacct

SEQ ID NO: 45 - DNA, 988 bp, synthetic construct
  source 1..988: mol_type = other DNA
catgattacgaattcagatctcgatcccgcgaaattaatacgactcactatagggagaccacaacggtttccctctagaaataattttgtttaactttaagaaggagatataccaatggtttcaaaaggtgaagaactgttcaccggggtggtgcccatcctggtcgagctggacggcgacgtaaacggccacaagttcagcgtgtccggcgagggcgagggcgatgccacctacggcaagctgaccctgaagttcatctgcaccaccggcaagctgcccgtgccctggcccaccctcgtgaccaccctgacctacggcgtgcagtgcttcagccgctaccccgaccacatgaagcagcacgacttcttcaagtccgccatgcccgaaggctacgtccaggagcgcaccatcttcttcaaggacgacggcaactacaagacccgcgccgaggtgaagttcgagggcgacaccctggtgaaccgcatcgagctgaagggcatcgacttcaaggaggacggcaacatcctggggcacaagctggagtacaactacaacagccacaacgtctatatcatggccgacaagcagaagaacggcatcaaggtgaacttcaagatccgccacaacatcgaggacggcagcgtgcagctcgccgaccactaccagcagaacacccccatcggcgacggccccgtgctgctgcccgacaaccactacctgagcacccagtccgccctgagcaaagaccccaacgagaagcgcgatcacatggtcctgctggagttcgtgaccgccgccgggatcactctcggcatggacgagctgtacaagggtggttcaagatggccattatggatgtggtttgtttggggttcacatcatcatcatcatcattaataattgattgatctagcataaccccttggggcctctaaacgggtcttgaggggttttttgctgaaaggaggaactatatccggataacct

SEQ ID NO: 46 - protein, 11 aa, synthetic construct
CRWPLWMWFVW

SEQ ID NO: 47 - protein, 19 aa, synthetic construct
CGKEGGSRWLIFHYMLLGG

SEQ ID NO: 48 - protein, 11 aa, synthetic construct
CRYYAHWLHYM

SEQ ID NO: 49 - protein, 11 aa, synthetic construct
CLFKAWLGVYH

SEQ ID NO: 50 - protein, 14 aa, synthetic construct
CGGSRVVSYLAEYH

SEQ ID NO: 51 - protein, 12 aa, synthetic construct
CYGRKKRRQRRR

SEQ ID NO: 52 - RNA, 21 nt, synthetic construct
  source 1..21: mol_type = other RNA
cttacgctgagtacttcgatt

SEQ ID NO: 53 - RNA, 21 nt, synthetic construct
  source 1..21: mol_type = other RNA
tcgaagtactcagcgtaagtt

SEQ ID NO: 54 - protein, 11 aa, synthetic construct
CTVTRGERYKH

SEQ ID NO: 55 - protein, 11 aa, synthetic construct
CMNYHKSNRHN

SEQ ID NO: 56 - protein, 11 aa, synthetic construct
CVRVKTYWENH